European Patent Application EP 4 266 314 A2, published October 25, 2023. Title: Error Suppression In Sequenced Dna Fragments Using Redundant Reads With Unique Molecular Indices (UMIs). Applicant: ILLUMINA. Application EP 0000000000.0, filed April 20, 2016. The sequence listing filed with the application follows.

SEQUENCE LISTING (3 sequences)

SEQ ID NO: 1 - skipped

SEQ ID NO: 2 - DNA, 45 bp, synthetic construct
  misc_feature 1..45: note = Synthetic polynucleotide
  misc_feature 1..4: note = n is a, c, g, or t
  source 1..45: mol_type = other DNA
nnnntgctcgcagatcggaagagcacacgtctgaactccagtcac

SEQ ID NO: 3 - DNA, 44 bp, synthetic construct
  misc_feature 1..44: note = Synthetic polynucleotide
  misc_feature 40..43: note = n is a, c, g, or t
  source 1..44: mol_type = other DNA
cactctttccctacacgacgctcttccgatctgcgaccannnnt